European Patent Specification EP 3 897 669 B1, published May 20, 2026. Title: METHODS AND COMPOSITIONS RELATED TO THERAPEUTIC PEPTIDES FOR CANCER THERAPY. Applicant: The University of Chicago. The sequence listing filed with the application follows.

SEQUENCE LISTING (5 sequences)

SEQ ID NO: 1 - protein, 335 aa, Homo sapiens
MLGIWTLLPLVLTSVARLSSKSVNAQVTDINSKGLELRKTVTTVETQNLEGLHHDGQFCHKPCPPGERKARDCTVNGDEPDCVPCQEGKEYTDKAHFSSKCRRCRLCDEGHGLEVEINCTRTQNTKCRCKPNFFCNSTVCEHCDPCTKCEHGIIKECTLTSNTKCKEEGSRSNLGWLCLLLLPIPLIVWVKRKEVQKTCRKHRKENQGSHESPTLNPETVAINLSDVDLSKYITTIAGVMTLSQVKGFVRKNGVNEAKIDEIKNDNVQDTAEQKVQLLRNWHQLHGKKEAYDTLIKDLKKANLCTLAEKIQTIILKDITSDSENSNFRNEIQSLV

SEQ ID NO: 2 - protein, 124 aa, Artificial Sequence
  Synthetic peptide
SPTLNPETVAINLSDVDLSKYITTIAGVMTLSQVKGFVRKNGVNEAKIDEIKNDNVQDTAEQKVQLLRNWHQLHGKKEAYDTLIKDLKKANLCTLAEKIQTIILKDITSDSENSNFRNEIQSLV

SEQ ID NO: 3 - protein, 115 aa, Artificial Sequence
  Synthetic peptide
AINLSDVDLSKYITTIAGVMTLSQVKGFVRKNGVNEAKIDEIKNDNVQDTAEQKVQLLRNWHQLHGKKEAYDTLIKDLKKANLCTLAEKIQTIILKDITSDSENSNFRNEIQSLV

SEQ ID NO: 4 - protein, 120 aa, Artificial Sequence
  Synthetic peptide
SPTLNPETVAINLSDVDLSKYITTIAGVMTLSQVKGFVRKNGVNEAKIDEIKNDNVQDTAEQKVQLLRNWHQLHGKKEAYDTLIKDLKKANLCTLAEKIQTIILKDITSDSENSNFRNEI

SEQ ID NO: 5 - protein, 111 aa, Artificial Sequence
  Synthetic peptide
AINLSDVDLSKYITTIAGVMTLSQVKGFVRKNGVNEAKIDEIKNDNVQDTAEQKVQLLRNWHQLHGKKEAYDTLIKDLKKANLCTLAEKIQTIILKDITSDSENSNFRNEI